European Patent Application EP 4 620 971 A1, published September 24, 2025. Title: T-CELL RECEPTORS RECOGNIZING NEORIBOEPITOPES. Applicant: ERVIMMUNE. The sequence listing filed with the application follows.

SEQUENCE LISTING (32 sequences)

SEQ ID NO: 1 - protein, 9 aa, synthetic construct
YSDRGSQSF

SEQ ID NO: 2 - protein, 6 aa, synthetic construct
IYSNGD

SEQ ID NO: 3 - protein, 11 aa, synthetic construct
CAVTNAGKSTF

SEQ ID NO: 4 - protein, 9 aa, synthetic construct
SPRSGDLSV

SEQ ID NO: 5 - protein, 18 aa, synthetic construct
QYYNGEERAKGNILERFS

SEQ ID NO: 6 - protein, 17 aa, synthetic construct
CASSFPLGGGRVDTQYF

SEQ ID NO: 7 - DNA, 27 bp, synthetic construct
  source 1..27: mol_type = other DNA
tacagtgaccgaggttcccagtccttc

SEQ ID NO: 8 - DNA, 18 bp, synthetic construct
  source 1..18: mol_type = other DNA
atatactccaatggtgac

SEQ ID NO: 9 - DNA, 33 bp, synthetic construct
  source 1..33: mol_type = other DNA
tgtgccgttacgaatgcaggcaaatcaaccttt

SEQ ID NO: 10 - DNA, 27 bp, synthetic construct
  source 1..27: mol_type = other DNA
tcccctaggtctggagacctctctgtg

SEQ ID NO: 11 - DNA, 54 bp, synthetic construct
  source 1..54: mol_type = other DNA
cagtattataatggagaagagagagcaaaaggaaacattcttgaacgattctcc

SEQ ID NO: 12 - DNA, 51 bp, synthetic construct
  source 1..51: mol_type = other DNA
tgtgccagcagcttccctctggggggcgggagagtggatacgcagtatttt

SEQ ID NO: 13 - protein, 9 aa, synthetic construct
LLLEATANL

SEQ ID NO: 14 - protein, 131 aa, synthetic construct
MKSLRVLLVILWLQLSWVWSQQKEVEQNSGPLSVPEGAIASLNCTYSDRGSQSFFWYRQYSGKSPELIMSIYSNGDKEDGRFTAQLNKASQYVSLLIRDSQPSDSATYLCAVTNAGKSTFGDGTTLTVKPN

SEQ ID NO: 15 - protein, 135 aa, synthetic construct
MGFRLLCCVAFCLLGAGPVDSGVTQTPKHLITATGQRVTLRCSPRSGDLSVYWYQQSLDQGLQFLIQYYNGEERAKGNILERFSAQQFPDLHSELNLSSLELGDSALYFCASSFPLGGGRVDTQYFGPGTRLTVL

SEQ ID NO: 16 - DNA, 393 bp, synthetic construct
  source 1..393: mol_type = other DNA
atgaaatccttgagagttttactagtgatcctgtggcttcagttgagctgggtttggagccaacagaaggaggtggagcagaattctggacccctcagtgttccagagggagccattgcctctctcaactgcacttacagtgaccgaggttcccagtccttcttctggtacagacaatattctgggaaaagccctgagttgataatgtccatatactccaatggtgacaaagaagatggaaggtttacagcacagctcaataaagccagccagtatgtttctctgctcatcagagactcccagcccagtgattcagccacctacctctgtgccgttacgaatgcaggcaaatcaacctttggggatgggactacgctcactgtgaagccaaat

SEQ ID NO: 17 - DNA, 405 bp, synthetic construct
  source 1..405: mol_type = other DNA
atgggcttcaggctcctctgctgtgtggccttttgtctcctgggagcaggcccagtggattctggagtcacacaaaccccaaagcacctgatcacagcaactggacagcgagtgacgctgagatgctcccctaggtctggagacctctctgtgtactggtaccaacagagcctggaccagggcctccagttcctcattcagtattataatggagaagagagagcaaaaggaaacattcttgaacgattctccgcacaacagttccctgacttgcactctgaactaaacctgagctctctggagctgggggactcagctttgtatttctgtgccagcagcttccctctggggggcgggagagtggatacgcagtattttggcccaggcacccggctgacagtgctc

SEQ ID NO: 18 - protein, 136 aa, synthetic construct
IQNPEPAVYQLKDPRSQDSTLCLFTDFDSQINVPKTMESGTFITDKTVLDMKAMDSKSNGAIAWSNQTSFTCQDIFKETNATYPSSDVPCDATLTEKSFETDMNLNFQNLSVMGLRILLLKVAGFNLLMTLRLWSS

SEQ ID NO: 19 - protein, 173 aa, synthetic construct
EDLRNVTPPKVSLFEPSKAEIANKQKATLVCLARGFFPDHVELSWWVNGKEVHSGVSTDPQAYKESNYSYCLSSRLRVSATFWHNPRNHFRCQVQFHGLSEEDKWPEGSPKPVTQNISAEAWGRADCGITSASYHQGVLSATILYEILLGKATLYAVLVSGLVLMAMVKKKNS

SEQ ID NO: 20 - protein, 136 aa, synthetic construct
IQNPEPAVYQLKDPRSQDSTLCLFTDFDSQINVPKTMESGTFITDKCVLDMKAMDSKSNGAIAWSNQTSFTCQDIFKETNATYPSSDVPCDATLTEKSFETDMNLNFQNLSVMGLRILLLKVAGFNLLMTLRLWSS

SEQ ID NO: 21 - protein, 173 aa, synthetic construct
EDLRNVTPPKVSLFEPSKAEIANKQKATLVCLARGFFPDHVELSWWVNGKEVHSGVCTDPQAYKESNYSYCLSSRLRVSATFWHNPRNHFRCQVQFHGLSEEDKWPEGSPKPVTQNISAEAWGRADCGITSASYHQGVLSATILYEILLGKATLYAVLVSGLVLMAMVKKKNS

SEQ ID NO: 22 - protein, 140 aa, synthetic construct
IQNPDPAVYQLRDSKSSDKSVCLFTDFDSQTNVSQSKDSDVYITDKTVLDMRSMDFKSNSAVAWSNKSDFACANAFNNSIIPEDTFFPSPESSCDVKLVEKSFETDTNLNFQNLSVIGFRILLLKVAGFNLLMTLRLWSS

SEQ ID NO: 23 - protein, 177 aa, synthetic construct
EDLKNVFPPEVAVFEPSEAEISHTQKATLVCLATGFFPDHVELSWWVNGKEVHSGVSTDPQPLKEQPALNDSRYCLSSRLRVSATFWQNPRNHFRCQVQFYGLSENDEWTQDRAKPVTQIVSAEAWGRADCGFTSVSYQQGVLSATILYEILLGKATLYAVLVSALVLMAMVKRKDF

SEQ ID NO: 24 - protein, 140 aa, synthetic construct
IQNPDPAVYQLRDSKSSDKSVCLFTDFDSQTNVSQSKDSDVYITDKCVLDMRSMDFKSNSAVAWSNKSDFACANAFNNSIIPEDTFFPSPESSCDVKLVEKSFETDTNLNFQNLSVIGFRILLLKVAGFNLLMTLRLWSS

SEQ ID NO: 25 - protein, 177 aa, synthetic construct
EDLKNVFPPEVAVFEPSEAEISHTQKATLVCLATGFFPDHVELSWWVNGKEVHSGVCTDPQPLKEQPALNDSRYCLSSRLRVSATFWQNPRNHFRCQVQFYGLSENDEWTQDRAKPVTQIVSAEAWGRADCGFTSVSYQQGVLSATILYEILLGKATLYAVLVSALVLMAMVKRKDF

SEQ ID NO: 26 - protein, 6 aa, synthetic construct
DRGSQS

SEQ ID NO: 27 - protein, 9 aa, synthetic construct
AVTNAGKST

SEQ ID NO: 28 - protein, 5 aa, synthetic construct
SGDLS

SEQ ID NO: 29 - protein, 6 aa, synthetic construct
YYNGEE

SEQ ID NO: 30 - protein, 15 aa, synthetic construct
ASSFPLGGGRVDTQY

SEQ ID NO: 31 - protein, 5 aa, synthetic construct
DKTVL

SEQ ID NO: 32 - protein, 5 aa, synthetic construct
GVSTD